European Patent Specification EP 3 621 642 B1, published September 18, 2024. Title: HUMAN MONOCLONAL ANTIBODIES AGAINST LAG3 AND USES THEREOF. Applicant: SMET PHARMACEUTICAL INC CHEN, Weizao XIAO, Zuoxiang FU, Tao. Application Unassigned. The sequence listing filed with the application follows.

SEQUENCE LISTING (113 sequences)

SEQ ID NO: 1 - protein, 110 aa, Artificial Sequence
  Human IgG variable domain with mutants
QSVLTQPPSVSAAPGRKVTISCSGSSSNIGTNSVSWYQQFPGTAPKLLIYDNNKRLSRIPDRFSGSKSGTSASLAISGLQSEDEADYYCAAWDDSLTGYVFGTGTKVTVL

SEQ ID NO: 2 - protein, 107 aa, Artificial Sequence
  Human IgG variable domain with mutants
DIQLTQSPSSLSASVGDRVTITCRASQNIGTYLNWYQQKPGKAPKLLIYAASSLQSGVPSRFSGSGSGTDFTLTISSLQPEDFATYYCQQLNSYPITFGQGTRLEIK

SEQ ID NO: 3 - protein, 110 aa, Artificial Sequence
  Human IgG variable domain with mutants
QSVLTQPPSVSAAPGQKVTISCSGSTSNIAINYVSWYQQVPGTVPKLLIYDDDKRPSGIPDRFSGSKSGTSATLDISGLQTGDEAHYYCGVWDNSLLAVLFGGGTSLTVL

SEQ ID NO: 4 - protein, 113 aa, Artificial Sequence
  Human IgG variable domain with mutants
DIQLTQSPDSLAVSLGERATINCKSSQSVLYSSNNKNYLAWYQQKPGQPPKLLIYWASTRESGVPDRFSGSGSGTDFTLTISSLQAEDVAVYYCQQYYSTPFTFGPGTKVDIK

SEQ ID NO: 5 - protein, 107 aa, Artificial Sequence
  Human IgG variable domain with mutants
DIQMTQSPSSLSASVGDRVTITCQASQDISNYLNWYQQKPGKAPKLLIYAASILQSGVPSRFSGSGSGTDFTLTISSLQPEDFATYYCQQSHSYSETFGQGTKVEIK

SEQ ID NO: 6 - protein, 111 aa, Artificial Sequence
  Human IgG variable domain with mutants
QSVVTQPPSVSGAPGQRVTVSCTGSSSNIGADFDVHWYQQLPGTAPKLLIYGNTNRPSGVPDRFSGSKSGTSASLAITGLQAEDEADYYCQSYDNSLSGVVFGGGTKVTVL

SEQ ID NO: 7 - protein, 107 aa, Artificial Sequence
  Human IgG variable domain with mutants
DIQLTQSPSSLSASVGDRVTITCRASRRISSYLNWYQQKQGKAPQLLIYAASSLQSGVPSRFSGSGSGTEFTLTISSLQPEDFATYYCQQFNSYPLTFGGGTKVEIK

SEQ ID NO: 8 - protein, 216 aa, Artificial Sequence
  Human IgG with mutants
QSVLTQPPSVSAAPGQKVTISCSGSTSNIAINYVSWYQQVPGTVPKLLIYDDDKRPSGIPDRFSGSKSGTSATLDISGLQTGDEAHYYCGVWDNSLLAVLFGGGTSLTVLGQPKAAPSVTLFPPSSEELQANKATLVCLISDFYPGAVTVAWKADSSPVKAGVETTTPSKQSNNKYAASSYLSLTPEQWKSHRSYSCQVTHEGSTVEKTVAPTECS

SEQ ID NO: 9 - protein, 118 aa, Artificial Sequence
  Human IgG variable domain with mutants
QVQLQQWGAGLLKPSETLSLTCAVYGGSFSGYYWSWIRQPPGKGLEWIGEINHSGSTNYNPSLKSRVTISVDTSKNQFSLKLSSVTAADTAVYYCARITPRFDAFDIWGQGTMVTVSS

SEQ ID NO: 10 - protein, 115 aa, Artificial Sequence
  Human IgG variable domain with mutants
EVQLVQSGAEVKKPGASVKVSCKASGGTFSSYTISWVRQAPGQGLEWMGGIIPIFGTANYAQKFQGRVTITADKSTSTAYMELSSLRSEDTAVYYCARDPVFDYWGQGTLVTVSS

SEQ ID NO: 11 - protein, 121 aa, Artificial Sequence
  Human IgG variable domain with mutants
EVQLVQSGAEVKKPGASVKVSCKASGYTFTSYGISWVRQAPGQGLEWMGWISAYNGNTNYAQKLQGRVTMTTDTSTSTAYMELRSLRSDDTAVYYCARDSSSWWVDAFDIWGQGTMVTVSS

SEQ ID NO: 12 - protein, 121 aa, Artificial Sequence
  Human IgG variable domain with mutants
EVQLVQSGAEVKKPGSSVKVSCKASGGTFSSYAISWVRQAPGQGLEWMGGIIPIFGTANYAQKFQGRVTITADESTSTAYMELSSLRSEDTAVYYCAREKPTGGYYGMDVWGKGTLVTVSS

SEQ ID NO: 13 - protein, 124 aa, Artificial Sequence
  Human IgG variable domain with mutants
QVQLVQSGAEVKKPGASVKVSCKASGGTFSSYAISWVRQAPGQGLEWMGGIIPIFGTANYAQKFQGRVTITADESTSTAYMELSSLRSEDTAVYYCARASPPAAYYYYYGMDVWGQGTTVTVSS

SEQ ID NO: 14 - protein, 126 aa, Artificial Sequence
  Human IgG variable domain with mutants
EVQLVQSGAEVKKPGESLKISCKGSGYSFTSYWIGWVRQMPGKGLEWMGIIYPGDSDTRYSPSFQGQVTISADKSISTAYLQWSSLKASDTAMYYCASGAPGYYYDSSGYYAFDIWGQGTMVTVSS

SEQ ID NO: 15 - protein, 121 aa, Artificial Sequence
  Human IgG variable domain with mutants
EVQLVESGAEVKKPGSSVKVSCKASGGTFSSYAISWVRQAPGQGLEWMGGIIPIFGTANYAQKFQGRVTITADKSTSTAYMELSSLRSEDTAVYYCALDGKSGFDLAFDIWGQGTMVTVSS

SEQ ID NO: 16 - protein, 451 aa, Artificial Sequence
  Human IgG with mutants
EVQLVQSGAEVKKPGASVKVSCKASGYTFTSYGISWVRQAPGQGLEWMGWISAYNGNTNYAQKLQGRVTMTTDTSTSTAYMELRSLRSDDTAVYYCARDSSSWWVDAFDIWGQGTMVTVSSASTKGPSVFPLAPSSKSTSGGTAALGCLVKDYFPEPVTVSWNSGALTSGVHTFPAVLQSSGLYSLSSVVTVPSSSLGTQTYICNVNHKPSNTKVDKKVEPKSCDKTHTCPPCPAPELLGGPSVFLFPPKPKDTLMISRTPEVTCVVVDVSHEDPEVKFNWYVDGVEVHNAKTKPREEQYNSTYRVVSVLTVLHQDWLNGKEYKCKVSNKALPAPIEKTISKAKGQPREPQVYTLPPSRDELTKNQVSLTCLVKGFYPSDIAVEWESNGQPENNYKTTPPVLDSDGSFFLYSKLTVDKSRWQQGNVFSCSVMHEALHNHYTQKSLSLSPGK

SEQ ID NO: 17 - protein, 448 aa, Artificial Sequence
  Human IgG with mutants
EVQLVQSGAEVKKPGASVKVSCKASGYTFTSYGISWVRQAPGQGLEWMGWISAYNGNTNYAQKLQGRVTMTTDTSTSTAYMELRSLRSDDTAVYYCARDSSSWWVDAFDIWGQGTMVTVSSASTKGPSVFPLAPCSRSTSESTAALGCLVKDYFPEPVTVSWNSGALTSGVHTFPAVLQSSGLYSLSSVVTVPSSSLGTKTYTCNVDHKPSNTKVDKRVESKYGPPCPPCPAPEFLGGPSVFLFPPKPKDTLMISRTPEVTCVVVDVSQEDPEVQFNWYVDGVEVHNAKTKPREEQFNSTYRVVSVLTVLHQDWLNGKEYKCKVSNKGLPSSIEKTISKAKGQPREPQVYTLPPSQEEMTKNQVSLTCLVKGFYPSDIAVEWESNGQPENNYKTTPPVLDSDGSFFLYSRLTVDKSRWQEGNVFSCSVMHEALHNHYTQKSLSLSLGK

SEQ ID NO: 18 - protein, 8 aa, Artificial Sequence
  Human IgG CDR with mutants
SSNIGTNS

SEQ ID NO: 19 - protein, 6 aa, Artificial Sequence
  Human IgG CDR with mutants
QNIGTY

SEQ ID NO: 20 - protein, 8 aa, Artificial Sequence
  Human IgG CDR with mutants
TSNIAINY

SEQ ID NO: 21 - protein, 12 aa, Artificial Sequence
  Human IgG CDR with mutants
QSVLYSSNNKNY

SEQ ID NO: 22 - protein, 6 aa, Artificial Sequence
  Human IgG CDR with mutants
QDISNY

SEQ ID NO: 23 - protein, 9 aa, Artificial Sequence
  Human IgG CDR with mutants
SSNIGADFD

SEQ ID NO: 24 - protein, 6 aa, Artificial Sequence
  Human IgG CDR with mutants
RRISSY

SEQ ID NO: 25 - protein, 11 aa, Artificial Sequence
  Human IgG CDR with mutants
AAWDDSLTGYV

SEQ ID NO: 26 - protein, 9 aa, Artificial Sequence
  Human IgG CDR with mutants
QQLNSYPIT

SEQ ID NO: 27 - protein, 11 aa, Artificial Sequence
  Human IgG CDR with mutants
GVWDNSLLAVL

SEQ ID NO: 28 - protein, 9 aa, Artificial Sequence
  Human IgG CDR with mutants
QQYYSTPFT

SEQ ID NO: 29 - protein, 9 aa, Artificial Sequence
  Human IgG CDR with mutants
QQSHSYSET

SEQ ID NO: 30 - protein, 11 aa, Artificial Sequence
  Human IgG CDR with mutants
QSYDNSLSGVV

SEQ ID NO: 31 - protein, 9 aa, Artificial Sequence
  Human IgG CDR with mutants
QQFNSYPLT

SEQ ID NO: 32 - protein, 8 aa, Artificial Sequence
  Human IgG CDR with mutants
GGSFSGYY

SEQ ID NO: 33 - protein, 8 aa, Artificial Sequence
  Human IgG CDR with mutants
GGTFSSYT

SEQ ID NO: 34 - protein, 8 aa, Artificial Sequence
  Human IgG CDR with mutants
GYTFTSYG

SEQ ID NO: 35 - protein, 8 aa, Artificial Sequence
  Human IgG CDR with mutants
GGTFSSYA

SEQ ID NO: 36 - protein, 8 aa, Artificial Sequence
  Human IgG CDR with mutants
GGTFSSYA

SEQ ID NO: 37 - protein, 8 aa, Artificial Sequence
  Human IgG CDR with mutants
GYSFTSYW

SEQ ID NO: 38 - protein, 8 aa, Artificial Sequence
  Human IgG CDR with mutants
GGTFSSYA

SEQ ID NO: 39 - protein, 7 aa, Artificial Sequence
  Human IgG CDR with mutants
INHSGST

SEQ ID NO: 40 - protein, 8 aa, Artificial Sequence
  Human IgG CDR with mutants
IIPIFGTA

SEQ ID NO: 41 - protein, 8 aa, Artificial Sequence
  Human IgG CDR with mutants
ISAYNGNT

SEQ ID NO: 42 - protein, 8 aa, Artificial Sequence
  Human IgG CDR with mutants
IIPIFGTA

SEQ ID NO: 43 - protein, 8 aa, Artificial Sequence
  Human IgG CDR with mutants
IIPIFGTA

SEQ ID NO: 44 - protein, 8 aa, Artificial Sequence
  Human IgG CDR with mutants
IYPGDSDT

SEQ ID NO: 45 - protein, 8 aa, Artificial Sequence
  Human IgG CDR with mutants
IIPIFGTA

SEQ ID NO: 46 - protein, 12 aa, Artificial Sequence
  Human IgG CDR with mutants
ARITPRFDAFDI

SEQ ID NO: 47 - protein, 8 aa, Artificial Sequence
  Human IgG CDR with mutants
ARDPVFDY

SEQ ID NO: 48 - protein, 14 aa, Artificial Sequence
  Human IgG CDR with mutants
ARDSSSWWVDAFDI

SEQ ID NO: 49 - protein, 14 aa, Artificial Sequence
  Human IgG CDR with mutants
AREKPTGGYYGMDV

SEQ ID NO: 50 - protein, 17 aa, Artificial Sequence
  Human IgG CDR with mutants
ARASPPAAYYYYYGMDV

SEQ ID NO: 51 - protein, 19 aa, Artificial Sequence
  Human IgG CDR with mutants
ASGAPGYYYDSSGYYAFDI

SEQ ID NO: 52 - protein, 14 aa, Artificial Sequence
  Human IgG CDR with mutants
ALDGKSGFDLAFDI

SEQ ID NO: 53 - protein, 8 aa, Artificial Sequence
  Human IgG CDR with mutants
SSNIGGNS

SEQ ID NO: 54 - protein, 8 aa, Artificial Sequence
  Human IgG CDR with mutants
SSNIGRNI

SEQ ID NO: 55 - protein, 8 aa, Artificial Sequence
  Human IgG CDR with mutants
SSNIGNNA

SEQ ID NO: 56 - protein, 8 aa, Artificial Sequence
  Human IgG CDR with mutants
GSNLQSNT

SEQ ID NO: 57 - protein, 8 aa, Artificial Sequence
  Human IgG CDR with mutants
TSNIGGNT

SEQ ID NO: 58 - protein, 8 aa, Artificial Sequence
  Human IgG CDR with mutants
SSNIGSNA

SEQ ID NO: 59 - protein, 8 aa, Artificial Sequence
  Human IgG CDR with mutants
RSNIGNNA

SEQ ID NO: 60 - protein, 8 aa, Artificial Sequence
  Human IgG CDR with mutants
SSNIASNA

SEQ ID NO: 61 - protein, 8 aa, Artificial Sequence
  Human IgG CDR with mutants
SSNIGSNI

SEQ ID NO: 62 - protein, 8 aa, Artificial Sequence
  Human IgG CDR with mutants
YSNIGGNT

SEQ ID NO: 63 - protein, 8 aa, Artificial Sequence
  Human IgG CDR with mutants
SSNIASNA

SEQ ID NO: 64 - protein, 8 aa, Artificial Sequence
  Human IgG CDR with mutants
SSNIGSAT

SEQ ID NO: 65 - protein, 8 aa, Artificial Sequence
  Human IgG CDR with mutants
SSNIASNA

SEQ ID NO: 66 - protein, 8 aa, Artificial Sequence
  Human IgG CDR with mutants
SSNIGNNA

SEQ ID NO: 67 - protein, 11 aa, Artificial Sequence
  Human IgG CDR with mutants
AAWDDSLNAYV

SEQ ID NO: 68 - protein, 12 aa, Artificial Sequence
  Human IgG CDR with mutants
AAWDDSLNGHML

SEQ ID NO: 69 - protein, 12 aa, Artificial Sequence
  Human IgG CDR with mutants
AAWDDSLSGQVL

SEQ ID NO: 70 - protein, 11 aa, Artificial Sequence
  Human IgG CDR with mutants
AAWDDRLDAYV

SEQ ID NO: 71 - protein, 11 aa, Artificial Sequence
  Human IgG CDR with mutants
AAWDDSLIAYV

SEQ ID NO: 72 - protein, 11 aa, Artificial Sequence
  Human IgG CDR with mutants
AAWDDSLNAFV

SEQ ID NO: 73 - protein, 11 aa, Artificial Sequence
  Human IgG CDR with mutants
AAWDDSLNGVL

SEQ ID NO: 74 - protein, 11 aa, Artificial Sequence
  Human IgG CDR with mutants
AAWDDSLNGVL

SEQ ID NO: 75 - protein, 12 aa, Artificial Sequence
  Human IgG CDR with mutants
AVWDDSLDGHLL

SEQ ID NO: 76 - protein, 11 aa, Artificial Sequence
  Human IgG CDR with mutants
AAWDDNLNGLV

SEQ ID NO: 77 - protein, 11 aa, Artificial Sequence
  Human IgG CDR with mutants
AAWDDSLNGVL

SEQ ID NO: 78 - protein, 11 aa, Artificial Sequence
  Human IgG CDR with mutants
AAWDGSLDGVM

SEQ ID NO: 79 - protein, 11 aa, Artificial Sequence
  Human IgG CDR with mutants
AAWDDSLNGVL

SEQ ID NO: 80 - protein, 11 aa, Artificial Sequence
  Human IgG CDR with mutants
AAWDDSLNAVV

SEQ ID NO: 81 - protein, 110 aa, Artificial Sequence
  Human IgG variable domain with mutants
LPVLTQPPSASGTPGQRVTISCSGSSSNIGGNSVNWYQQLPGTAPKLLIYSDNQRPSGVPDRFSGSKSGTSASLAISGLQSEEEADYYCAAWDDSLNAYVFGPGTKVTVL

SEQ ID NO: 82 - protein, 111 aa, Artificial Sequence
  Human IgG variable domain with mutants
SYELTQPPSASGTPGQRVTISCSGSSSNIGRNIVNWYQHLPGTAPKLLIYGNSQRPSGVPDRFSGSKSGTSASLAISGLQSEDEADYYCAAWDDSLNGHMLFGGGTKLTVL

SEQ ID NO: 83 - protein, 111 aa, Artificial Sequence
  Human IgG variable domain with mutants
QSVLTQPPSASGTPGQRVTISCSGSSSNIGNNAVNWYQQLPGKAPKLLIYYDDLLPSGVSDRFSGSKSGTSASLAISGLRSEDEGDYFCAAWDDSLSGQVLFGGGTKLTVL

SEQ ID NO: 84 - protein, 110 aa, Artificial Sequence
  Human IgG variable domain with mutants
SYVLTQPPSTSAAPGQTVTILCFGGGSNLQSNTVNWYRHVSGSAPKLLIHSDDERASGVSPRLSGSKSGGSASLILRGLQPEDEGDYYCAAWDDRLDAYVFGTGTKVTVL

SEQ ID NO: 85 - protein, 110 aa, Artificial Sequence
  Human IgG variable domain with mutants
QSVLTQPPSASGTPGQRVTISCSGSTSNIGGNTVNWYQQLPGTAPKLLIYSSNRRPSGVPDRFSGSTSGTSASLAISGLQSEDEADYYCAAWDDSLIAYVFGTGTKVTVL

SEQ ID NO: 86 - protein, 110 aa, Artificial Sequence
  Human IgG variable domain with mutants
SYELTQPPSVSEAPRQRVTISCSGSSSNIGSNAVSWYQQVPRKAPKLLVYYDDLLPSGVSDRFSGSKSGTSASLAIRGLQSEDEADYYCAAWDDSLNAFVFGTGTKVTVL

SEQ ID NO: 87 - protein, 110 aa, Artificial Sequence
  Human IgG variable domain with mutants
SYELTQPPSVSEAPRQRATISCSGSRSNIGNNAVSWYQRLPGQAPKLLIYYDTFLPSGVSDRFSGSKSGTSASLTISGLQSDDEADYYCAAWDDSLNGVLFGGGTKLTVQ

SEQ ID NO: 88 - protein, 110 aa, Artificial Sequence
  Human IgG variable domain with mutants
LPVLTQPPSVSGAPRQRVTISCSGGSSNIASNAVNWYQQFPGKAPKLLVYYDDLLPSGVSDRFSGSKTGTSASLAISALQSEDEADYFCAAWDDSLNGVLFGGGTKLTVL

SEQ ID NO: 89 - protein, 111 aa, Artificial Sequence
  Human IgG variable domain with mutants
SYVLTQPPSASGTPGQRVTISCSGSSSNIGSNIVNWYQHLPGTAPKLLIYGNSQRPSGVSDRFSGSKSGTSASLAISGLQSEDEANYYCAVWDDSLDGHLLFGGGTKLTVL

SEQ ID NO: 90 - protein, 110 aa, Artificial Sequence
  Human IgG variable domain with mutants
SYVLTQPPSASGTPGQRVTMSCSGRYSNIGGNTVNWYHHLPGTAPTLLIYSNDQRPSGVPDRFSGSKSGTSASLAISGVQSEDEADYYCAAWDDNLNGLVFGTGTKVTVL

SEQ ID NO: 91 - protein, 110 aa, Artificial Sequence
  Human IgG variable domain with mutants
PYVLTQPPSVSGAPRQRVTISCSGGSSNIASNAVNWYQQFPGKAPKLLVYYDDLLPSGVSDRFSGSKTGTSASLAISALQSEDEADYFCAAWDDSLNGVLFGGGTKLTVL

SEQ ID NO: 92 - protein, 110 aa, Artificial Sequence
  Human IgG variable domain with mutants
LPVLTQPPSASGTPGQRITISCSGSSSNIGSATVNWYQHLPGTAPKLLIYGDNQRPSGVADRFSGSKSGTSASLEIRGLQSEDEADYYCAAWDGSLDGVMFGGGTRVNVL

SEQ ID NO: 93 - protein, 110 aa, Artificial Sequence
  Human IgG variable domain with mutants
SYVLTQPPSASGTPGQRVTISCSGGSSNIASNAVNWYQQFPGKAPKLLVYYDDLLPSGVSDRFSGSKTGTSASLAISALQSEDEADYFCAAWDDSLNGVLFGGGTKLTVL

SEQ ID NO: 94 - protein, 109 aa, Artificial Sequence
  Human IgG variable domain with mutants
SVVTQPPSVSEAPRQRVTISCSGSSSNIGNNAVNWYQQLPGKAPKLLIYYDDLLPSGVSDRFSGSKSGTSASLAISGLQSEDEADYYCAAWDDSLNAVVFGGGTKLTVL

SEQ ID NO: 95 - DNA, 46 bp, Artificial Sequence
  Oligo primer
gtgtaagcttaccatgggtgtgcccactcaggtcctggggttgctg

SEQ ID NO: 96 - DNA, 46 bp, Artificial Sequence
  Oligo primer
gtgttctagagccgccaccatggaatggagctgggtctttctcttc

SEQ ID NO: 97 - DNA, 30 bp, Artificial Sequence
  Oligo primer
gatgccagatgtcagtctgtgttgacgcag

SEQ ID NO: 98 - DNA, 39 bp, Artificial Sequence
  Oligo primer
gccagagaatcggtcaggaatccctgagggtcgcttatc

SEQ ID NO: 99 - DNA, 18 bp, Artificial Sequence
  Oligo primer
cctgaccgattctctggc

SEQ ID NO: 100 - DNA, 31 bp, Artificial Sequence
  Oligo primer
gatcgaattcttatgaacattctgtaggggc

SEQ ID NO: 101 - DNA, 30 bp, Artificial Sequence
  Oligo primer
ggtgtccactccgaggtccagctggtgcag

SEQ ID NO: 102 - DNA, 29 bp, Artificial Sequence
  Oligo primer
gaagctgagctcacggtgaccattgtccc

SEQ ID NO: 103 - DNA, 32 bp, Artificial Sequence
  Oligo primer
gatcgagctcagcttccaccaagggcccatcc

SEQ ID NO: 104 - DNA, 36 bp, Artificial Sequence
  Oligo primer
cggccgtcgcactcatttacccagagacagggagag

SEQ ID NO: 105 - DNA, 18 bp, Artificial Sequence
  Oligo primer
tgagtgcgacggccggca

SEQ ID NO: 106 - DNA, 18 bp, Artificial Sequence
  Oligo primer
cccgaggtcgacgctctc

SEQ ID NO: 107 - protein, 216 aa, Artificial Sequence
  Human IgG with mutants
SYELTQPPSVSEAPRQRVTISCSGSSSNIGSNAVSWYQQVPRKAPKLLVYYDDLLPSGVSDRFSGSKSGTSASLAIRGLQSEDEADYYCAAWDDSLNAFVFGTGTKVTVLGQPKANPTVTLFPPSSEELQANKATLVCLISDFYPGAVTVAWKADGSPVKAGVETTKPSKQSNNKYAASSYLSLTPEQWKSHRSYSCQVTHEGSTVEKTVAPTECS

SEQ ID NO: 108 - protein, 216 aa, Artificial Sequence
  Human IgG with mutants
SYVLTQPPSASGTPGQRVTMSCSGRYSNIGGNTVNWYHHLPGTAPTLLIYSNDQRPSGVPDRFSGSKSGTSASLAISGVQSEDEADYYCAAWDDNLNGLVFGTGTKVTVLGQPKANPTVTLFPPSSEELQANKATLVCLISDFYPGAVTVAWKADGSPIKAGVETTKPSKQSNNKYAASSYLSLTPEQWKSHRSYSCQVTHEGSTVEKTVAPTECS

SEQ ID NO: 109 - protein, 215 aa, Artificial Sequence
  Human IgG with mutants
SVVTQPPSVSEAPRQRVTISCSGSSSNIGNNAVNWYQQLPGKAPKLLIYYDDLLPSGVSDRFSGSKSGTSASLAISGLQSEDEADYYCAAWDDSLNAVVFGGGTKLTVLGQPKAAPSVTLFPPSSEELQANKATLVCLISDFYPGAVTVAWKADSSPVKAGVETTTPSKQSNNKYAASSYLSLTPEQWKSHKSYSCQVTHEGSTVEKTVAPTECS

SEQ ID NO: 110 - DNA, 30 bp, Artificial Sequence
  Oligo primer
gatgccagatgttcctatgagctgactcag

SEQ ID NO: 111 - DNA, 31 bp, Artificial Sequence; identical to SEQ ID NO: 100
  Oligo primer

SEQ ID NO: 112 - DNA, 30 bp, Artificial Sequence
  Oligo primer
gatgccagatgttcctatgtgctgactcag

SEQ ID NO: 113 - DNA, 30 bp, Artificial Sequence
  Oligo primer
gatgccagatgttctgtcgtgacgcagccg